European Patent Application EP 4 464 175 A1, published November 20, 2024. Title: COMPOSITION FOR IMPROVING MEMORY OR COGNITION ABILITY, OR PREVENTING OR TREATING BRAIN NEUROLOGICAL DISEASES, COMPRISING PORCINE BRAIN ENZYME HYDROLYSATE. Applicant: UNIMED PHARMACEUTICALS INC. The sequence listing filed with the application follows.

SEQUENCE LISTING (2 sequences)

SEQ ID NO: 1 - protein, 4 aa, synthetic construct
  REGION 1..4: note = brPEP-1
PSIS

SEQ ID NO: 2 - protein, 9 aa, synthetic construct
  REGION 1..9: note = brPEP-2
GPAGPQGPR